European Patent Application EP 4 800 033 A1, published September 2, 2026. Title: ヒト化抗CKAP4抗体又はその抗原結合性断片. Applicant: 国立大学法人大阪大学. The sequence listing filed with the application follows.

SEQUENCE LISTING (31 sequences)

SEQ ID NO: 1 - protein, 10 aa, synthetic construct
GFTFTSYWMH

SEQ ID NO: 2 - protein, 20 aa, synthetic construct
WIGNINPSNGGTNYNAKFKS

SEQ ID NO: 3 - protein, 14 aa, synthetic construct
ARWVSFSYRGAMDY

SEQ ID NO: 4 - protein, 121 aa, synthetic construct
QVQLVQSGAEVKKPGASVKVSCKASGFTFTSYWMHWVRQAPGQGLEWIGNINPSNGGTNYNAKFKSRVTMTRDTSTSTVYMELSSLRSEDTAVYYCARWVSFSYRGAMDYWGQGTLVTVSS

SEQ ID NO: 5 - protein, 468 aa, synthetic construct
MDWTWRVFCLLAVAPGAHSQVQLVQSGAEVKKPGASVKVSCKASGFTFTSYWMHWVRQAPGQGLEWIGNINPSNGGTNYNAKFKSRVTMTRDTSTSTVYMELSSLRSEDTAVYYCARWVSFSYRGAMDYWGQGTLVTVSSASTKGPSVFPLAPSSKSTSGGTAALGCLVKDYFPEPVTVSWNSGALTSGVHTFPAVLQSSGLYSLSSVVTVPSSSLGTQTYICNVNHKPSNTKVDKKVEPKSCDKTHTCPPCPAPELLGGPSVFLFPPKPKDTLMISRTPEVTCVVVDVSHEDPEVKFNWYVDGVEVHNAKTKPREEQYNSTYRVVSVLTVLHQDWLNGKEYKCKVSNKALPAPIEKTISKAKGQPREPQVYTLPPSRDELTKNQVSLTCLVKGFYPSDIAVEWESNGQPENNYKTTPPVLDSDGSFFLYSKLTVDKSRWQQGNVFSCSVMHEALHNHYTQKSLSLSP

SEQ ID NO: 6 - protein, 5 aa, synthetic construct
SYWMH

SEQ ID NO: 7 - protein, 8 aa, synthetic construct
INPSNGGT

SEQ ID NO: 8 - protein, 12 aa, synthetic construct
WVSFSYRGAMDY

SEQ ID NO: 9 - protein, 121 aa, synthetic construct
QVQLVQSGAEVKKPGASVKVSCKASGYTFTSYWMHWVRQAPGQGLEWMGIINPSNGGTSYAQKFQGRVTMTRDTSTSTVYMELSSLRSEDTAVYYCARWVSFSYRGAMDYWGQGTLVTVSS

SEQ ID NO: 10 - protein, 468 aa, synthetic construct
MDWTWRVFCLLAVAPGAHSQVQLVQSGAEVKKPGASVKVSCKASGYTFTSYWMHWVRQAPGQGLEWMGIINPSNGGTSYAQKFQGRVTMTRDTSTSTVYMELSSLRSEDTAVYYCARWVSFSYRGAMDYWGQGTLVTVSSASTKGPSVFPLAPSSKSTSGGTAALGCLVKDYFPEPVTVSWNSGALTSGVHTFPAVLQSSGLYSLSSVVTVPSSSLGTQTYICNVNHKPSNTKVDKKVEPKSCDKTHTCPPCPAPELLGGPSVFLFPPKPKDTLMISRTPEVTCVVVDVSHEDPEVKFNWYVDGVEVHNAKTKPREEQYNSTYRVVSVLTVLHQDWLNGKEYKCKVSNKALPAPIEKTISKAKGQPREPQVYTLPPSRDELTKNQVSLTCLVKGFYPSDIAVEWESNGQPENNYKTTPPVLDSDGSFFLYSKLTVDKSRWQQGNVFSCSVMHEALHNHYTQKSLSLSP

SEQ ID NO: 11 - protein, 11 aa, synthetic construct
RASRAIRNNLH

SEQ ID NO: 12 - protein, 11 aa, synthetic construct
LLIKYVSQSIS

SEQ ID NO: 13 - protein, 9 aa, synthetic construct
QQSDSWPYT

SEQ ID NO: 14 - protein, 107 aa, synthetic construct
EIVLTQSPDFQSVTPKEKVTITCRASRAIRNNLHWYQQKPDQSPKLLIKYVSQSISGVPSRFSGSGSGTDFTLTINSLEAEDAATYYCQQSDSWPYTFGQGTKLEIK

SEQ ID NO: 15 - protein, 233 aa, synthetic construct
MLPSQLIGFLLLWVPASRGEIVLTQSPDFQSVTPKEKVTITCRASRAIRNNLHWYQQKPDQSPKLLIKYVSQSISGVPSRFSGSGSGTDFTLTINSLEAEDAATYYCQQSDSWPYTFGQGTKLEIKRTVAAPSVFIFPPSDEQLKSGTASVVCLLNNFYPREAKVQWKVDNALQSGNSQESVTEQDSKDSTYSLSSTLTLSKADYEKHKVYACEVTHQGLSSPVTKSFNRGEC

SEQ ID NO: 16 - protein, 328 aa, synthetic construct
ASTKGPSVFPLAPSSKSTSGGTAALGCLVKDYFPEPVTVSWNSGALTSGVHTFPAVLQSSGLYSLSSVVTVPSSSLGTQTYICNVNHKPSNTKVDKKVEPKSCDKTHTCPPCPAPELLGGPSVFLFPPKPKDTLMISRTPEVTCVVVDVSHEDPEVKFNWYVDGVEVHNAKTKPREEQYNSTYRVVSVLTVLHQDWLNGKEYKCKVSNKALPAPIEKTISKAKGQPREPQVYTLPPSRDELTKNQVSLTCLVKGFYPSDIAVEWESNGQPENNYKTTPPVLDSDGSFFLYSKLTVDKSRWQQGNVFSCSVMHEALHNHYTQKSLSLSP

SEQ ID NO: 17 - protein, 107 aa, synthetic construct [sequence omitted]

SEQ ID NO: 18 - DNA, 1407 bp, synthetic construct
  source 1..1407: mol_type = other DNA
atggattggacctggcgggtgttctgtctgctggctgttgctcctggcgctcactctcaggttcagctggttcagtctggcgccgaagtgaagaaacctggcgcctctgtgaaggtgtcctgcaaggcttccggcttcaccttcaccagctactggatgcactgggtccgacaggctccaggacaaggcttggagtggatcggcaacatcaacccttctaacggcggcaccaactacaacgccaagttcaagtccagagtgaccatgaccagagacacctccaccagcaccgtgtacatggaactgtccagcctgagatccgaggacaccgccgtgtactactgtgccagatgggtgtccttcagctataggggcgccatggattattggggccagggcacactggtcaccgtgtcatctgcctccaccaagggaccctctgtgtttcctctggctccctccagcaagtctacctctggtggaacagctgccctgggctgcctggtcaaggattactttcctgagcctgtgaccgtgtcctggaactctggcgctctgacatctggcgtgcacacctttccagctgtgctgcagtcctccggcctgtactctctgtcctctgtcgtgaccgtgccttccagctctctgggcacccagacctacatctgcaatgtgaaccacaagccttccaacaccaaggtggacaagaaggtggaacccaagtcctgcgacaagacccacacctgtcctccatgtcctgctccagaactgctcggcggaccttccgtgttcctgtttcctccaaagcctaaggacaccctgatgatctctcggacccctgaagtgacctgcgtggtggtggatgtgtctcacgaggatcccgaagtgaagttcaattggtacgtggacggcgtggaagtgcacaacgccaagaccaagcctagagaggaacagtacaactccacctacagagtggtgtccgtgctgaccgtgctgcaccaggattggctgaacggcaaagagtacaagtgcaaggtgtccaacaaggccctgcctgctcctatcgaaaagaccatctccaaggccaagggccagcctagggaaccccaggtttacaccttgcctccatctcgggacgagctgaccaagaaccaggtgtccctgacctgtctcgtgaagggcttctacccctccgatatcgccgtggaatgggagtctaatggccagcctgagaacaactacaagacaacccctcctgtgctggactccgacggctcattcttcctgtactccaagctgacagtggacaagtccagatggcagcagggcaacgtgttctcctgctccgtgatgcacgaggccctgcacaatcactacacccagaagtccctgtctctgtccccttga

SEQ ID NO: 19 - DNA, 1407 bp, synthetic construct
  source 1..1407: mol_type = other DNA
atggattggacctggcgggtgttctgtctgctggctgttgctcctggcgctcactctcaggttcagctggttcagtctggcgccgaagtgaagaaacctggcgcctctgtgaaggtgtcctgcaaggcttccggctacacctttaccagctactggatgcactgggtccgacaggctccaggacaaggcttggagtggatgggcatcatcaacccttctaacggcggcaccagctacgcccagaaattccagggcagagtgaccatgaccagagacacctccaccagcaccgtgtacatggaactgtccagcctgagatccgaggacaccgccgtgtactactgtgccagatgggtgtccttcagctataggggcgccatggattattggggccagggcacactggtcaccgtgtcatctgcctccaccaagggaccctctgtgtttcctctggctccctccagcaagtctacctctggtggaacagctgccctgggctgcctggtcaaggattactttcctgagcctgtgaccgtgtcctggaactctggcgctctgacatctggcgtgcacacctttccagctgtgctgcagtcctccggcctgtactctctgtcctctgtcgtgaccgtgccttccagctctctgggcacccagacctacatctgcaatgtgaaccacaagccttccaacaccaaggtggacaagaaggtggaacccaagtcctgcgacaagacccacacctgtcctccatgtcctgctccagaactgctcggcggaccttccgtgttcctgtttcctccaaagcctaaggacaccctgatgatctctcggacccctgaagtgacctgcgtggtggtggatgtgtctcacgaggatcccgaagtgaagttcaattggtacgtggacggcgtggaagtgcacaacgccaagaccaagcctagagaggaacagtacaactccacctacagagtggtgtccgtgctgaccgtgctgcaccaggattggctgaacggcaaagagtacaagtgcaaggtgtccaacaaggccctgcctgctcctatcgaaaagaccatctccaaggccaagggccagcctagggaaccccaggtttacaccttgcctccatctcgggacgagctgaccaagaaccaggtgtccctgacctgtctcgtgaagggcttctacccctccgatatcgccgtggaatgggagtctaatggccagcctgagaacaactacaagacaacccctcctgtgctggactccgacggctcattcttcctgtactccaagctgacagtggacaagtccagatggcagcagggcaacgtgttctcctgctccgtgatgcacgaggccctgcacaatcactacacccagaagtccctgtctctgtccccttga

SEQ ID NO: 20 - DNA, 702 bp, synthetic construct
  source 1..702: mol_type = other DNA
atgctgccctctcagctgatcggctttctgctgctgtgggtgccagcttccagaggcgagattgtgctgacccagtctcctgacttccagagcgtgacccctaaagagaaagtcaccatcacctgtcgggcctctcgggccatcagaaacaacctgcactggtatcagcaaaaacctgatcagtcccctaagctgctgatcaaatacgtgtcccagtccatctccggcgtgccctctagattttccggctctggctctggcaccgacttcaccctgaccatcaattccctggaagccgaggatgccgccacctactactgccagcagtctgactcttggccctacacctttggccagggcaccaagctggaaatcaagcgaacagtggctgccccttccgtgttcatcttcccaccttccgacgagcagctgaagtctggcacagcctctgtcgtgtgcctgctgaacaacttctaccctcgggaagccaaggtgcagtggaaggtggacaatgccctgcagtccggcaactcccaagagtctgtgaccgagcaggactccaaggacagcacctacagcctgtcctccacactgaccctgtccaaggccgactacgagaagcacaaggtgtacgcctgcgaagtgacccatcagggcctgtctagccctgtgaccaagtctttcaaccggggcgagtgctga

SEQ ID NO: 21 - DNA, 366 bp, synthetic construct
  source 1..366: mol_type = other DNA
caggtccaattgcagcagcagcctgggactgaactggtgaagcctggggcttcagtgaagctgtcttgcaaggcctctggcttcaccttcaccagctactggatgcactgggtaaaacagaggcctggacaaggccttgagtggattggaaatattaatcctagcaatggtggtactaactacaatgcgaagttcaagagtaaggccacactgactgtagacaaatcctccagtacagcctacatgcaactcagcagcctgacatctgaggactctgcggtctattattgtgcaagatgggtctcctttagttaccgaggggctatggactactggggtcaaggaacctcagtcaccgtctcctca

SEQ ID NO: 22 - protein, 122 aa, synthetic construct
QVQLQQQPGTELVKPGASVKLSCKASGFTFTSYWMHWVKQRPGQGLEWIGNINPSNGGTNYNAKFKSKATLTVDKSSSTAYMQLSSLTSEDSAVYYCARWVSFSYRGAMDYWGQGTSVTVSS

SEQ ID NO: 23 - DNA, 321 bp, synthetic construct
  source 1..321: mol_type = other DNA
gatattgtgctaactcagtctccagccattctgtctgtgactccaggagatggcgtcagtctttcctgcagggccagtcgagctattaggaacaacctacactggtttcaacaaaaatcacatgagtctccaaggcttctcatcaagtatgtttcccagtccatctctgggattccctccaggttcagtggcagtggatcagggacagatttcactctcagtgtcgacagtgtagagactgaagattttggagtgtatttctgtcaacagagtgacagctggccttacacgttcggaggggggaccaaactggaaataaaa

SEQ ID NO: 24 - protein, 107 aa, synthetic construct
DIVLTQSPAILSVTPGDGVSLSCRASRAIRNNLHWFQQKSHESPRLLIKYVSQSISGIPSRFSGSGSGTDFTLSVDSVETEDFGVYFCQQSDSWPYTFGGGTKLEIK

SEQ ID NO: 25 - protein, 602 aa, Homo sapiens
MPSAKQRGSKGGHGAASPSEKGAHPSGGADDVAKKPPPAPQQPPPPPAPHPQQHPQQHPQNQAHGKGGHRGGGGGGGKSSSSSSASAAAAAAAASSSASCSRRLGRALNFLFYLALVAAAAFSGWCVHHVLEEVQQVRRSHQDFSRQREELGQGLQGVEQKVQSLQATFGTFESILRSSQHKQDLTEKAVKQGESEVSRISEVLQKLQNEILKDLSDGIHVVKDARERDFTSLENTVEERLTELTKSINDNIAIFTEVQKRSQKEINDMKAKVASLEESEGNKQDLKALKEAVKEIQTSAKSREWDMEALRSTLQTMESDIYTEVRELVSLKQEQQAFKEAADTERLALQALTEKLLRSEESVSRLPEEIRRLEEELRQLKSDSHGPKEDGGFRHSEAFEALQQKSQGLDSRLQHVEDGVLSMQVASARQTESLESLLSKSQEHEQRLAALQGRLEGLGSSEADQDGLASTVRSLGETQLVLYGDVEELKRSVGELPSTVESLQKVQEQVHTLLSQDQAQAARLPPQDFLDRLSSLDNLKASVSQVEADLKMLRTAVDSLVAYSVKIETNENNLESAKGLLDDLRNDLDRLFVKVEKIHEKV

SEQ ID NO: 26 - DNA, 57 bp, synthetic construct
  source 1..57: mol_type = other DNA
atgggatggagctgtatcatcctctttctggtagcagcagctacaggtgtccactcc

SEQ ID NO: 27 - protein, 19 aa, synthetic construct
MGWSCIILFLVAAATGVHS

SEQ ID NO: 28 - DNA, 60 bp, synthetic construct
  source 1..60: mol_type = other DNA
atggttttcacacctcagatacttggacttatgcttttttggatttcagcctccagaggt

SEQ ID NO: 29 - protein, 20 aa, synthetic construct
MVFTPQILGLMLFWISASRG

SEQ ID NO: 30 - protein, 19 aa, synthetic construct
MDWTWRVFCLLAVAPGAHS

SEQ ID NO: 31 - protein, 19 aa, synthetic construct
MLPSQLIGFLLLWVPASRG